European Patent Application EP 4 116 424 A1, published January 11, 2023. Title: MODIFIED TRANSGLUTAMINASE. Applicant: AMANO ENZYME INC. The sequence listing filed with the application follows.

SEQUENCE LISTING (54 sequences)

SEQ ID NO: 1 - protein, 331 aa, Streptomyces mobaraensis
DSDDRVTPPAEPLDRMPDPYRPSYGRAETVVNNYIRKWQQVYSHRDGRKQQMTEEQREWLSYGCVGVTWVNSGQYPTNRLAFASFDEDRFKNELKNGRPRSGETRAEFEGRVAKESFDEEKGFQRAREVASVMNRALENAHDESAYLDNLKKELANGNDALRNEDARSPFYSALRNTPSFKERNGGNHDPSRMKAVIYSKHFWSGQDRSSSADKRKYGDPDAFRPAPGTGLVDMSRDRNIPRSPTSPGEGFVNFDYGWFGAQTEADADKTVWTHGNHYHAPNGSLGAMHVYESKFRNWSEGYSDFDRGAYVITFIPKSWNTAPDKVKQGWP

SEQ ID NO: 2 - protein, 331 aa, Artificial Sequence
  D3G mutant
DSGDRVTPPAEPLDRMPDPYRPSYGRAETVVNNYIRKWQQVYSHRDGRKQQMTEEQREWLSYGCVGVTWVNSGQYPTNRLAFASFDEDRFKNELKNGRPRSGETRAEFEGRVAKESFDEEKGFQRAREVASVMNRALENAHDESAYLDNLKKELANGNDALRNEDARSPFYSALRNTPSFKERNGGNHDPSRMKAVIYSKHFWSGQDRSSSADKRKYGDPDAFRPAPGTGLVDMSRDRNIPRSPTSPGEGFVNFDYGWFGAQTEADADKTVWTHGNHYHAPNGSLGAMHVYESKFRNWSEGYSDFDRGAYVITFIPKSWNTAPDKVKQGWP

SEQ ID NO: 3 - protein, 331 aa, Artificial Sequence
  D3K mutant
DSKDRVTPPAEPLDRMPDPYRPSYGRAETVVNNYIRKWQQVYSHRDGRKQQMTEEQREWLSYGCVGVTWVNSGQYPTNRLAFASFDEDRFKNELKNGRPRSGETRAEFEGRVAKESFDEEKGFQRAREVASVMNRALENAHDESAYLDNLKKELANGNDALRNEDARSPFYSALRNTPSFKERNGGNHDPSRMKAVIYSKHFWSGQDRSSSADKRKYGDPDAFRPAPGTGLVDMSRDRNIPRSPTSPGEGFVNFDYGWFGAQTEADADKTVWTHGNHYHAPNGSLGAMHVYESKFRNWSEGYSDFDRGAYVITFIPKSWNTAPDKVKQGWP

SEQ ID NO: 4 - protein, 331 aa, Artificial Sequence
  D3W mutant
DSWDRVTPPAEPLDRMPDPYRPSYGRAETVVNNYIRKWQQVYSHRDGRKQQMTEEQREWLSYGCVGVTWVNSGQYPTNRLAFASFDEDRFKNELKNGRPRSGETRAEFEGRVAKESFDEEKGFQRAREVASVMNRALENAHDESAYLDNLKKELANGNDALRNEDARSPFYSALRNTPSFKERNGGNHDPSRMKAVIYSKHFWSGQDRSSSADKRKYGDPDAFRPAPGTGLVDMSRDRNIPRSPTSPGEGFVNFDYGWFGAQTEADADKTVWTHGNHYHAPNGSLGAMHVYESKFRNWSEGYSDFDRGAYVITFIPKSWNTAPDKVKQGWP

SEQ ID NO: 5 - protein, 331 aa, Artificial Sequence
  D3G/F305W mutant
DSGDRVTPPAEPLDRMPDPYRPSYGRAETVVNNYIRKWQQVYSHRDGRKQQMTEEQREWLSYGCVGVTWVNSGQYPTNRLAFASFDEDRFKNELKNGRPRSGETRAEFEGRVAKESFDEEKGFQRAREVASVMNRALENAHDESAYLDNLKKELANGNDALRNEDARSPFYSALRNTPSFKERNGGNHDPSRMKAVIYSKHFWSGQDRSSSADKRKYGDPDAFRPAPGTGLVDMSRDRNIPRSPTSPGEGFVNFDYGWFGAQTEADADKTVWTHGNHYHAPNGSLGAMHVYESKFRNWSEGYSDWDRGAYVITFIPKSWNTAPDKVKQGWP

SEQ ID NO: 6 - protein, 331 aa, Artificial Sequence
  D3K/F305W mutant
DSKDRVTPPAEPLDRMPDPYRPSYGRAETVVNNYIRKWQQVYSHRDGRKQQMTEEQREWLSYGCVGVTWVNSGQYPTNRLAFASFDEDRFKNELKNGRPRSGETRAEFEGRVAKESFDEEKGFQRAREVASVMNRALENAHDESAYLDNLKKELANGNDALRNEDARSPFYSALRNTPSFKERNGGNHDPSRMKAVIYSKHFWSGQDRSSSADKRKYGDPDAFRPAPGTGLVDMSRDRNIPRSPTSPGEGFVNFDYGWFGAQTEADADKTVWTHGNHYHAPNGSLGAMHVYESKFRNWSEGYSDWDRGAYVITFIPKSWNTAPDKVKQGWP

SEQ ID NO: 7 - protein, 331 aa, Artificial Sequence
  D3N/F305W mutant
DSNDRVTPPAEPLDRMPDPYRPSYGRAETVVNNYIRKWQQVYSHRDGRKQQMTEEQREWLSYGCVGVTWVNSGQYPTNRLAFASFDEDRFKNELKNGRPRSGETRAEFEGRVAKESFDEEKGFQRAREVASVMNRALENAHDESAYLDNLKKELANGNDALRNEDARSPFYSALRNTPSFKERNGGNHDPSRMKAVIYSKHFWSGQDRSSSADKRKYGDPDAFRPAPGTGLVDMSRDRNIPRSPTSPGEGFVNFDYGWFGAQTEADADKTVWTHGNHYHAPNGSLGAMHVYESKFRNWSEGYSDWDRGAYVITFIPKSWNTAPDKVKQGWP

SEQ ID NO: 8 - protein, 331 aa, Artificial Sequence
  D3P/F305W mutant
DSPDRVTPPAEPLDRMPDPYRPSYGRAETVVNNYIRKWQQVYSHRDGRKQQMTEEQREWLSYGCVGVTWVNSGQYPTNRLAFASFDEDRFKNELKNGRPRSGETRAEFEGRVAKESFDEEKGFQRAREVASVMNRALENAHDESAYLDNLKKELANGNDALRNEDARSPFYSALRNTPSFKERNGGNHDPSRMKAVIYSKHFWSGQDRSSSADKRKYGDPDAFRPAPGTGLVDMSRDRNIPRSPTSPGEGFVNFDYGWFGAQTEADADKTVWTHGNHYHAPNGSLGAMHVYESKFRNWSEGYSDWDRGAYVITFIPKSWNTAPDKVKQGWP

SEQ ID NO: 9 - protein, 331 aa, Artificial Sequence
  D3W/F305W mutant
DSWDRVTPPAEPLDRMPDPYRPSYGRAETVVNNYIRKWQQVYSHRDGRKQQMTEEQREWLSYGCVGVTWVNSGQYPTNRLAFASFDEDRFKNELKNGRPRSGETRAEFEGRVAKESFDEEKGFQRAREVASVMNRALENAHDESAYLDNLKKELANGNDALRNEDARSPFYSALRNTPSFKERNGGNHDPSRMKAVIYSKHFWSGQDRSSSADKRKYGDPDAFRPAPGTGLVDMSRDRNIPRSPTSPGEGFVNFDYGWFGAQTEADADKTVWTHGNHYHAPNGSLGAMHVYESKFRNWSEGYSDWDRGAYVITFIPKSWNTAPDKVKQGWP

SEQ ID NO: 10 - protein, 331 aa, Artificial Sequence
  Y34W/F305W mutant
DSDDRVTPPAEPLDRMPDPYRPSYGRAETVVNNWIRKWQQVYSHRDGRKQQMTEEQREWLSYGCVGVTWVNSGQYPTNRLAFASFDEDRFKNELKNGRPRSGETRAEFEGRVAKESFDEEKGFQRAREVASVMNRALENAHDESAYLDNLKKELANGNDALRNEDARSPFYSALRNTPSFKERNGGNHDPSRMKAVIYSKHFWSGQDRSSSADKRKYGDPDAFRPAPGTGLVDMSRDRNIPRSPTSPGEGFVNFDYGWFGAQTEADADKTVWTHGNHYHAPNGSLGAMHVYESKFRNWSEGYSDWDRGAYVITFIPKSWNTAPDKVKQGWP

SEQ ID NO: 11 - protein, 331 aa, Artificial Sequence
  V65I/F305W mutant
DSDDRVTPPAEPLDRMPDPYRPSYGRAETVVNNYIRKWQQVYSHRDGRKQQMTEEQREWLSYGCIGVTWVNSGQYPTNRLAFASFDEDRFKNELKNGRPRSGETRAEFEGRVAKESFDEEKGFQRAREVASVMNRALENAHDESAYLDNLKKELANGNDALRNEDARSPFYSALRNTPSFKERNGGNHDPSRMKAVIYSKHFWSGQDRSSSADKRKYGDPDAFRPAPGTGLVDMSRDRNIPRSPTSPGEGFVNFDYGWFGAQTEADADKTVWTHGNHYHAPNGSLGAMHVYESKFRNWSEGYSDWDRGAYVITFIPKSWNTAPDKVKQGWP

SEQ ID NO: 12 - protein, 331 aa, Artificial Sequence
  S303K/F305W mutant
DSDDRVTPPAEPLDRMPDPYRPSYGRAETVVNNYIRKWQQVYSHRDGRKQQMTEEQREWLSYGCVGVTWVNSGQYPTNRLAFASFDEDRFKNELKNGRPRSGETRAEFEGRVAKESFDEEKGFQRAREVASVMNRALENAHDESAYLDNLKKELANGNDALRNEDARSPFYSALRNTPSFKERNGGNHDPSRMKAVIYSKHFWSGQDRSSSADKRKYGDPDAFRPAPGTGLVDMSRDRNIPRSPTSPGEGFVNFDYGWFGAQTEADADKTVWTHGNHYHAPNGSLGAMHVYESKFRNWSEGYKDWDRGAYVITFIPKSWNTAPDKVKQGWP

SEQ ID NO: 13 - protein, 331 aa, Artificial Sequence
  S303R/F305W mutant
DSDDRVTPPAEPLDRMPDPYRPSYGRAETVVNNYIRKWQQVYSHRDGRKQQMTEEQREWLSYGCVGVTWVNSGQYPTNRLAFASFDEDRFKNELKNGRPRSGETRAEFEGRVAKESFDEEKGFQRAREVASVMNRALENAHDESAYLDNLKKELANGNDALRNEDARSPFYSALRNTPSFKERNGGNHDPSRMKAVIYSKHFWSGQDRSSSADKRKYGDPDAFRPAPGTGLVDMSRDRNIPRSPTSPGEGFVNFDYGWFGAQTEADADKTVWTHGNHYHAPNGSLGAMHVYESKFRNWSEGYRDWDRGAYVITFIPKSWNTAPDKVKQGWP

SEQ ID NO: 14 - protein, 331 aa, Artificial Sequence
  R5H mutant
DSDDHVTPPAEPLDRMPDPYRPSYGRAETVVNNYIRKWQQVYSHRDGRKQQMTEEQREWLSYGCVGVTWVNSGQYPTNRLAFASFDEDRFKNELKNGRPRSGETRAEFEGRVAKESFDEEKGFQRAREVASVMNRALENAHDESAYLDNLKKELANGNDALRNEDARSPFYSALRNTPSFKERNGGNHDPSRMKAVIYSKHFWSGQDRSSSADKRKYGDPDAFRPAPGTGLVDMSRDRNIPRSPTSPGEGFVNFDYGWFGAQTEADADKTVWTHGNHYHAPNGSLGAMHVYESKFRNWSEGYSDFDRGAYVITFIPKSWNTAPDKVKQGWP

SEQ ID NO: 15 - protein, 331 aa, Artificial Sequence
  V6D mutant
DSDDRDTPPAEPLDRMPDPYRPSYGRAETVVNNYIRKWQQVYSHRDGRKQQMTEEQREWLSYGCVGVTWVNSGQYPTNRLAFASFDEDRFKNELKNGRPRSGETRAEFEGRVAKESFDEEKGFQRAREVASVMNRALENAHDESAYLDNLKKELANGNDALRNEDARSPFYSALRNTPSFKERNGGNHDPSRMKAVIYSKHFWSGQDRSSSADKRKYGDPDAFRPAPGTGLVDMSRDRNIPRSPTSPGEGFVNFDYGWFGAQTEADADKTVWTHGNHYHAPNGSLGAMHVYESKFRNWSEGYSDFDRGAYVITFIPKSWNTAPDKVKQGWP

SEQ ID NO: 16 - protein, 331 aa, Artificial Sequence
  W59T mutant
DSDDRVTPPAEPLDRMPDPYRPSYGRAETVVNNYIRKWQQVYSHRDGRKQQMTEEQRETLSYGCVGVTWVNSGQYPTNRLAFASFDEDRFKNELKNGRPRSGETRAEFEGRVAKESFDEEKGFQRAREVASVMNRALENAHDESAYLDNLKKELANGNDALRNEDARSPFYSALRNTPSFKERNGGNHDPSRMKAVIYSKHFWSGQDRSSSADKRKYGDPDAFRPAPGTGLVDMSRDRNIPRSPTSPGEGFVNFDYGWFGAQTEADADKTVWTHGNHYHAPNGSLGAMHVYESKFRNWSEGYSDFDRGAYVITFIPKSWNTAPDKVKQGWP

SEQ ID NO: 17 - protein, 331 aa, Artificial Sequence
  S61G mutant
DSDDRVTPPAEPLDRMPDPYRPSYGRAETVVNNYIRKWQQVYSHRDGRKQQMTEEQREWLGYGCVGVTWVNSGQYPTNRLAFASFDEDRFKNELKNGRPRSGETRAEFEGRVAKESFDEEKGFQRAREVASVMNRALENAHDESAYLDNLKKELANGNDALRNEDARSPFYSALRNTPSFKERNGGNHDPSRMKAVIYSKHFWSGQDRSSSADKRKYGDPDAFRPAPGTGLVDMSRDRNIPRSPTSPGEGFVNFDYGWFGAQTEADADKTVWTHGNHYHAPNGSLGAMHVYESKFRNWSEGYSDFDRGAYVITFIPKSWNTAPDKVKQGWP

SEQ ID NO: 18 - protein, 331 aa, Artificial Sequence
  S61R mutant
DSDDRVTPPAEPLDRMPDPYRPSYGRAETVVNNYIRKWQQVYSHRDGRKQQMTEEQREWLRYGCVGVTWVNSGQYPTNRLAFASFDEDRFKNELKNGRPRSGETRAEFEGRVAKESFDEEKGFQRAREVASVMNRALENAHDESAYLDNLKKELANGNDALRNEDARSPFYSALRNTPSFKERNGGNHDPSRMKAVIYSKHFWSGQDRSSSADKRKYGDPDAFRPAPGTGLVDMSRDRNIPRSPTSPGEGFVNFDYGWFGAQTEADADKTVWTHGNHYHAPNGSLGAMHVYESKFRNWSEGYSDFDRGAYVITFIPKSWNTAPDKVKQGWP

SEQ ID NO: 19 - protein, 331 aa, Artificial Sequence
  M288F mutant
DSDDRVTPPAEPLDRMPDPYRPSYGRAETVVNNYIRKWQQVYSHRDGRKQQMTEEQREWLSYGCVGVTWVNSGQYPTNRLAFASFDEDRFKNELKNGRPRSGETRAEFEGRVAKESFDEEKGFQRAREVASVMNRALENAHDESAYLDNLKKELANGNDALRNEDARSPFYSALRNTPSFKERNGGNHDPSRMKAVIYSKHFWSGQDRSSSADKRKYGDPDAFRPAPGTGLVDMSRDRNIPRSPTSPGEGFVNFDYGWFGAQTEADADKTVWTHGNHYHAPNGSLGAFHVYESKFRNWSEGYSDFDRGAYVITFIPKSWNTAPDKVKQGWP

SEQ ID NO: 20 - protein, 331 aa, Artificial Sequence
  M288L mutant
DSDDRVTPPAEPLDRMPDPYRPSYGRAETVVNNYIRKWQQVYSHRDGRKQQMTEEQREWLSYGCVGVTWVNSGQYPTNRLAFASFDEDRFKNELKNGRPRSGETRAEFEGRVAKESFDEEKGFQRAREVASVMNRALENAHDESAYLDNLKKELANGNDALRNEDARSPFYSALRNTPSFKERNGGNHDPSRMKAVIYSKHFWSGQDRSSSADKRKYGDPDAFRPAPGTGLVDMSRDRNIPRSPTSPGEGFVNFDYGWFGAQTEADADKTVWTHGNHYHAPNGSLGALHVYESKFRNWSEGYSDFDRGAYVITFIPKSWNTAPDKVKQGWP

SEQ ID NO: 21 - protein, 331 aa, Artificial Sequence
  M288Y mutant
DSDDRVTPPAEPLDRMPDPYRPSYGRAETVVNNYIRKWQQVYSHRDGRKQQMTEEQREWLSYGCVGVTWVNSGQYPTNRLAFASFDEDRFKNELKNGRPRSGETRAEFEGRVAKESFDEEKGFQRAREVASVMNRALENAHDESAYLDNLKKELANGNDALRNEDARSPFYSALRNTPSFKERNGGNHDPSRMKAVIYSKHFWSGQDRSSSADKRKYGDPDAFRPAPGTGLVDMSRDRNIPRSPTSPGEGFVNFDYGWFGAQTEADADKTVWTHGNHYHAPNGSLGAYHVYESKFRNWSEGYSDFDRGAYVITFIPKSWNTAPDKVKQGWP

SEQ ID NO: 22 - protein, 331 aa, Artificial Sequence
  V290I mutant
DSDDRVTPPAEPLDRMPDPYRPSYGRAETVVNNYIRKWQQVYSHRDGRKQQMTEEQREWLSYGCVGVTWVNSGQYPTNRLAFASFDEDRFKNELKNGRPRSGETRAEFEGRVAKESFDEEKGFQRAREVASVMNRALENAHDESAYLDNLKKELANGNDALRNEDARSPFYSALRNTPSFKERNGGNHDPSRMKAVIYSKHFWSGQDRSSSADKRKYGDPDAFRPAPGTGLVDMSRDRNIPRSPTSPGEGFVNFDYGWFGAQTEADADKTVWTHGNHYHAPNGSLGAMHIYESKFRNWSEGYSDFDRGAYVITFIPKSWNTAPDKVKQGWP

SEQ ID NO: 23 - DNA, 1134 bp, Artificial Sequence
  D3G mutant
atggacaatggcgcgggggaagagacgaagtcctacgccgaaacctaccgcctcacggcggatgacgtcgcgaacatcaacgcgctcaacgaaagcgctccggccgcttcgagcgccggcccgtcgttccgggcccccgactccggcgacagggtcacccctcccgccgagccgctcgacaggatgcccgacccgtaccgtccctcgtacggcagggccgagacggtcgtcaacaactacatacgcaagtggcagcaggtctacagccaccgcgacggcaggaagcagcagatgaccgaggagcagcgggagtggctgtcctacggctgcgtcggtgtcacctgggtcaattcgggtcagtacccgacgaacagactggccttcgcgtccttcgacgaggacaggttcaagaacgagctgaagaacggcaggccccggtccggcgagacgcgggcggagttcgagggccgcgtcgcgaaggagagcttcgacgaggagaagggcttccagcgggcgcgtgaggtggcgtccgtcatgaacagggccctggagaacgcccacgacgagagcgcttacctcgacaacctcaagaaggaactggcgaacggcaacgacgccctgcgcaacgaggacgcccgttccccgttctactcggcgctgcggaacacgccgtccttcaaggagcggaacggaggcaatcacgacccgtccaggatgaaggccgtcatctactcgaagcacttctggagcggccaggaccggtcgagttcggccgacaagaggaagtacggcgacccggacgccttccgccccgccccgggcaccggcctggtcgacatgtcgagggacaggaacattccgcgcagccccaccagccccggtgagggattcgtcaatttcgactacggctggttcggcgcccagacggaagcggacgccgacaagaccgtctggacccacggaaatcactatcacgcgcccaatggcagcctgggtgccatgcatgtctacgagagcaagttccgcaactggtccgagggttactcggacttcgaccgcggagcctatgtgatcaccttcatccccaagagctggaacaccgcccccgacaaggtaaagcagggctggccgtga

SEQ ID NO: 24 - DNA, 1134 bp, Artificial Sequence
  D3K mutant
atggacaatggcgcgggggaagagacgaagtcctacgccgaaacctaccgcctcacggcggatgacgtcgcgaacatcaacgcgctcaacgaaagcgctccggccgcttcgagcgccggcccgtcgttccgggcccccgactccaaggacagggtcacccctcccgccgagccgctcgacaggatgcccgacccgtaccgtccctcgtacggcagggccgagacggtcgtcaacaactacatacgcaagtggcagcaggtctacagccaccgcgacggcaggaagcagcagatgaccgaggagcagcgggagtggctgtcctacggctgcgtcggtgtcacctgggtcaattcgggtcagtacccgacgaacagactggccttcgcgtccttcgacgaggacaggttcaagaacgagctgaagaacggcaggccccggtccggcgagacgcgggcggagttcgagggccgcgtcgcgaaggagagcttcgacgaggagaagggcttccagcgggcgcgtgaggtggcgtccgtcatgaacagggccctggagaacgcccacgacgagagcgcttacctcgacaacctcaagaaggaactggcgaacggcaacgacgccctgcgcaacgaggacgcccgttccccgttctactcggcgctgcggaacacgccgtccttcaaggagcggaacggaggcaatcacgacccgtccaggatgaaggccgtcatctactcgaagcacttctggagcggccaggaccggtcgagttcggccgacaagaggaagtacggcgacccggacgccttccgccccgccccgggcaccggcctggtcgacatgtcgagggacaggaacattccgcgcagccccaccagccccggtgagggattcgtcaatttcgactacggctggttcggcgcccagacggaagcggacgccgacaagaccgtctggacccacggaaatcactatcacgcgcccaatggcagcctgggtgccatgcatgtctacgagagcaagttccgcaactggtccgagggttactcggacttcgaccgcggagcctatgtgatcaccttcatccccaagagctggaacaccgcccccgacaaggtaaagcagggctggccgtga

SEQ ID NO: 25 - DNA, 1134 bp, Artificial Sequence
  D3W mutant
atggacaatggcgcgggggaagagacgaagtcctacgccgaaacctaccgcctcacggcggatgacgtcgcgaacatcaacgcgctcaacgaaagcgctccggccgcttcgagcgccggcccgtcgttccgggcccccgactcctgggacagggtcacccctcccgccgagccgctcgacaggatgcccgacccgtaccgtccctcgtacggcagggccgagacggtcgtcaacaactacatacgcaagtggcagcaggtctacagccaccgcgacggcaggaagcagcagatgaccgaggagcagcgggagtggctgtcctacggctgcgtcggtgtcacctgggtcaattcgggtcagtacccgacgaacagactggccttcgcgtccttcgacgaggacaggttcaagaacgagctgaagaacggcaggccccggtccggcgagacgcgggcggagttcgagggccgcgtcgcgaaggagagcttcgacgaggagaagggcttccagcgggcgcgtgaggtggcgtccgtcatgaacagggccctggagaacgcccacgacgagagcgcttacctcgacaacctcaagaaggaactggcgaacggcaacgacgccctgcgcaacgaggacgcccgttccccgttctactcggcgctgcggaacacgccgtccttcaaggagcggaacggaggcaatcacgacccgtccaggatgaaggccgtcatctactcgaagcacttctggagcggccaggaccggtcgagttcggccgacaagaggaagtacggcgacccggacgccttccgccccgccccgggcaccggcctggtcgacatgtcgagggacaggaacattccgcgcagccccaccagccccggtgagggattcgtcaatttcgactacggctggttcggcgcccagacggaagcggacgccgacaagaccgtctggacccacggaaatcactatcacgcgcccaatggcagcctgggtgccatgcatgtctacgagagcaagttccgcaactggtccgagggttactcggacttcgaccgcggagcctatgtgatcaccttcatccccaagagctggaacaccgcccccgacaaggtaaagcagggctggccgtga

SEQ ID NO: 26 - DNA, 1134 bp, Artificial Sequence
  D3G/F305W mutant
atggacaatggcgcgggggaagagacgaagtcctacgccgaaacctaccgcctcacggcggatgacgtcgcgaacatcaacgcgctcaacgaaagcgctccggccgcttcgagcgccggcccgtcgttccgggcccccgactccggcgacagggtcacccctcccgccgagccgctcgacaggatgcccgacccgtaccgtccctcgtacggcagggccgagacggtcgtcaacaactacatacgcaagtggcagcaggtctacagccaccgcgacggcaggaagcagcagatgaccgaggagcagcgggagtggctgtcctacggctgcgtcggtgtcacctgggtcaattcgggtcagtacccgacgaacagactggccttcgcgtccttcgacgaggacaggttcaagaacgagctgaagaacggcaggccccggtccggcgagacgcgggcggagttcgagggccgcgtcgcgaaggagagcttcgacgaggagaagggcttccagcgggcgcgtgaggtggcgtccgtcatgaacagggccctggagaacgcccacgacgagagcgcttacctcgacaacctcaagaaggaactggcgaacggcaacgacgccctgcgcaacgaggacgcccgttccccgttctactcggcgctgcggaacacgccgtccttcaaggagcggaacggaggcaatcacgacccgtccaggatgaaggccgtcatctactcgaagcacttctggagcggccaggaccggtcgagttcggccgacaagaggaagtacggcgacccggacgccttccgccccgccccgggcaccggcctggtcgacatgtcgagggacaggaacattccgcgcagccccaccagccccggtgagggattcgtcaatttcgactacggctggttcggcgcccagacggaagcggacgccgacaagaccgtctggacccacggaaatcactatcacgcgcccaatggcagcctgggtgccatgcatgtctacgagagcaagttccgcaactggtccgagggttactcggactgggaccgcggagcctatgtgatcaccttcatccccaagagctggaacaccgcccccgacaaggtaaagcagggctggccgtga

SEQ ID NO: 27 - DNA, 1134 bp, Artificial Sequence
  D3K/F305W mutant
atggacaatggcgcgggggaagagacgaagtcctacgccgaaacctaccgcctcacggcggatgacgtcgcgaacatcaacgcgctcaacgaaagcgctccggccgcttcgagcgccggcccgtcgttccgggcccccgactccaaggacagggtcacccctcccgccgagccgctcgacaggatgcccgacccgtaccgtccctcgtacggcagggccgagacggtcgtcaacaactacatacgcaagtggcagcaggtctacagccaccgcgacggcaggaagcagcagatgaccgaggagcagcgggagtggctgtcctacggctgcgtcggtgtcacctgggtcaattcgggtcagtacccgacgaacagactggccttcgcgtccttcgacgaggacaggttcaagaacgagctgaagaacggcaggccccggtccggcgagacgcgggcggagttcgagggccgcgtcgcgaaggagagcttcgacgaggagaagggcttccagcgggcgcgtgaggtggcgtccgtcatgaacagggccctggagaacgcccacgacgagagcgcttacctcgacaacctcaagaaggaactggcgaacggcaacgacgccctgcgcaacgaggacgcccgttccccgttctactcggcgctgcggaacacgccgtccttcaaggagcggaacggaggcaatcacgacccgtccaggatgaaggccgtcatctactcgaagcacttctggagcggccaggaccggtcgagttcggccgacaagaggaagtacggcgacccggacgccttccgccccgccccgggcaccggcctggtcgacatgtcgagggacaggaacattccgcgcagccccaccagccccggtgagggattcgtcaatttcgactacggctggttcggcgcccagacggaagcggacgccgacaagaccgtctggacccacggaaatcactatcacgcgcccaatggcagcctgggtgccatgcatgtctacgagagcaagttccgcaactggtccgagggttactcggactgggaccgcggagcctatgtgatcaccttcatccccaagagctggaacaccgcccccgacaaggtaaagcagggctggccgtga

SEQ ID NO: 28 - DNA, 1134 bp, Artificial Sequence
  D3N/F305W mutant
atggacaatggcgcgggggaagagacgaagtcctacgccgaaacctaccgcctcacggcggatgacgtcgcgaacatcaacgcgctcaacgaaagcgctccggccgcttcgagcgccggcccgtcgttccgggcccccgactccaacgacagggtcacccctcccgccgagccgctcgacaggatgcccgacccgtaccgtccctcgtacggcagggccgagacggtcgtcaacaactacatacgcaagtggcagcaggtctacagccaccgcgacggcaggaagcagcagatgaccgaggagcagcgggagtggctgtcctacggctgcgtcggtgtcacctgggtcaattcgggtcagtacccgacgaacagactggccttcgcgtccttcgacgaggacaggttcaagaacgagctgaagaacggcaggccccggtccggcgagacgcgggcggagttcgagggccgcgtcgcgaaggagagcttcgacgaggagaagggcttccagcgggcgcgtgaggtggcgtccgtcatgaacagggccctggagaacgcccacgacgagagcgcttacctcgacaacctcaagaaggaactggcgaacggcaacgacgccctgcgcaacgaggacgcccgttccccgttctactcggcgctgcggaacacgccgtccttcaaggagcggaacggaggcaatcacgacccgtccaggatgaaggccgtcatctactcgaagcacttctggagcggccaggaccggtcgagttcggccgacaagaggaagtacggcgacccggacgccttccgccccgccccgggcaccggcctggtcgacatgtcgagggacaggaacattccgcgcagccccaccagccccggtgagggattcgtcaatttcgactacggctggttcggcgcccagacggaagcggacgccgacaagaccgtctggacccacggaaatcactatcacgcgcccaatggcagcctgggtgccatgcatgtctacgagagcaagttccgcaactggtccgagggttactcggactgggaccgcggagcctatgtgatcaccttcatccccaagagctggaacaccgcccccgacaaggtaaagcagggctggccgtga

SEQ ID NO: 29 - DNA, 1134 bp, Artificial Sequence
  D3P/F305W mutant
atggacaatggcgcgggggaagagacgaagtcctacgccgaaacctaccgcctcacggcggatgacgtcgcgaacatcaacgcgctcaacgaaagcgctccggccgcttcgagcgccggcccgtcgttccgggcccccgactccccggacagggtcacccctcccgccgagccgctcgacaggatgcccgacccgtaccgtccctcgtacggcagggccgagacggtcgtcaacaactacatacgcaagtggcagcaggtctacagccaccgcgacggcaggaagcagcagatgaccgaggagcagcgggagtggctgtcctacggctgcgtcggtgtcacctgggtcaattcgggtcagtacccgacgaacagactggccttcgcgtccttcgacgaggacaggttcaagaacgagctgaagaacggcaggccccggtccggcgagacgcgggcggagttcgagggccgcgtcgcgaaggagagcttcgacgaggagaagggcttccagcgggcgcgtgaggtggcgtccgtcatgaacagggccctggagaacgcccacgacgagagcgcttacctcgacaacctcaagaaggaactggcgaacggcaacgacgccctgcgcaacgaggacgcccgttccccgttctactcggcgctgcggaacacgccgtccttcaaggagcggaacggaggcaatcacgacccgtccaggatgaaggccgtcatctactcgaagcacttctggagcggccaggaccggtcgagttcggccgacaagaggaagtacggcgacccggacgccttccgccccgccccgggcaccggcctggtcgacatgtcgagggacaggaacattccgcgcagccccaccagccccggtgagggattcgtcaatttcgactacggctggttcggcgcccagacggaagcggacgccgacaagaccgtctggacccacggaaatcactatcacgcgcccaatggcagcctgggtgccatgcatgtctacgagagcaagttccgcaactggtccgagggttactcggactgggaccgcggagcctatgtgatcaccttcatccccaagagctggaacaccgcccccgacaaggtaaagcagggctggccgtga

SEQ ID NO: 30 - DNA, 1134 bp, Artificial Sequence
  D3W/F305W mutant i
atggacaatggcgcgggggaagagacgaagtcctacgccgaaacctaccgcctcacggcggatgacgtcgcgaacatcaacgcgctcaacgaaagcgctccggccgcttcgagcgccggcccgtcgttccgggcccccgactcctgggacagggtcacccctcccgccgagccgctcgacaggatgcccgacccgtaccgtccctcgtacggcagggccgagacggtcgtcaacaactacatacgcaagtggcagcaggtctacagccaccgcgacggcaggaagcagcagatgaccgaggagcagcgggagtggctgtcctacggctgcgtcggtgtcacctgggtcaattcgggtcagtacccgacgaacagactggccttcgcgtccttcgacgaggacaggttcaagaacgagctgaagaacggcaggccccggtccggcgagacgcgggcggagttcgagggccgcgtcgcgaaggagagcttcgacgaggagaagggcttccagcgggcgcgtgaggtggcgtccgtcatgaacagggccctggagaacgcccacgacgagagcgcttacctcgacaacctcaagaaggaactggcgaacggcaacgacgccctgcgcaacgaggacgcccgttccccgttctactcggcgctgcggaacacgccgtccttcaaggagcggaacggaggcaatcacgacccgtccaggatgaaggccgtcatctactcgaagcacttctggagcggccaggaccggtcgagttcggccgacaagaggaagtacggcgacccggacgccttccgccccgccccgggcaccggcctggtcgacatgtcgagggacaggaacattccgcgcagccccaccagccccggtgagggattcgtcaatttcgactacggctggttcggcgcccagacggaagcggacgccgacaagaccgtctggacccacggaaatcactatcacgcgcccaatggcagcctgggtgccatgcatgtctacgagagcaagttccgcaactggtccgagggttactcggactgggaccgcggagcctatgtgatcaccttcatccccaagagctggaacaccgcccccgacaaggtaaagcagggctggccgtga

SEQ ID NO: 31 - DNA, 1134 bp, Artificial Sequence
  Y34W/F305W mutant
atggacaatggcgcgggggaagagacgaagtcctacgccgaaacctaccgcctcacggcggatgacgtcgcgaacatcaacgcgctcaacgaaagcgctccggccgcttcgagcgccggcccgtcgttccgggcccccgactccgacgacagggtcacccctcccgccgagccgctcgacaggatgcccgacccgtaccgtccctcgtacggcagggccgagacggtcgtcaacaactggatacgcaagtggcagcaggtctacagccaccgcgacggcaggaagcagcagatgaccgaggagcagcgggagtggctgtcctacggctgcgtcggtgtcacctgggtcaattcgggtcagtacccgacgaacagactggccttcgcgtccttcgacgaggacaggttcaagaacgagctgaagaacggcaggccccggtccggcgagacgcgggcggagttcgagggccgcgtcgcgaaggagagcttcgacgaggagaagggcttccagcgggcgcgtgaggtggcgtccgtcatgaacagggccctggagaacgcccacgacgagagcgcttacctcgacaacctcaagaaggaactggcgaacggcaacgacgccctgcgcaacgaggacgcccgttccccgttctactcggcgctgcggaacacgccgtccttcaaggagcggaacggaggcaatcacgacccgtccaggatgaaggccgtcatctactcgaagcacttctggagcggccaggaccggtcgagttcggccgacaagaggaagtacggcgacccggacgccttccgccccgccccgggcaccggcctggtcgacatgtcgagggacaggaacattccgcgcagccccaccagccccggtgagggattcgtcaatttcgactacggctggttcggcgcccagacggaagcggacgccgacaagaccgtctggacccacggaaatcactatcacgcgcccaatggcagcctgggtgccatgcatgtctacgagagcaagttccgcaactggtccgagggttactcggactgggaccgcggagcctatgtgatcaccttcatccccaagagctggaacaccgcccccgacaaggtaaagcagggctggccgtga

SEQ ID NO: 32 - DNA, 1134 bp, Artificial Sequence
  V65I/F305W mutant
atggacaatggcgcgggggaagagacgaagtcctacgccgaaacctaccgcctcacggcggatgacgtcgcgaacatcaacgcgctcaacgaaagcgctccggccgcttcgagcgccggcccgtcgttccgggcccccgactccgacgacagggtcacccctcccgccgagccgctcgacaggatgcccgacccgtaccgtccctcgtacggcagggccgagacggtcgtcaacaactacatacgcaagtggcagcaggtctacagccaccgcgacggcaggaagcagcagatgaccgaggagcagcgggagtggctgtcctacggctgcatcggtgtcacctgggtcaattcgggtcagtacccgacgaacagactggccttcgcgtccttcgacgaggacaggttcaagaacgagctgaagaacggcaggccccggtccggcgagacgcgggcggagttcgagggccgcgtcgcgaaggagagcttcgacgaggagaagggcttccagcgggcgcgtgaggtggcgtccgtcatgaacagggccctggagaacgcccacgacgagagcgcttacctcgacaacctcaagaaggaactggcgaacggcaacgacgccctgcgcaacgaggacgcccgttccccgttctactcggcgctgcggaacacgccgtccttcaaggagcggaacggaggcaatcacgacccgtccaggatgaaggccgtcatctactcgaagcacttctggagcggccaggaccggtcgagttcggccgacaagaggaagtacggcgacccggacgccttccgccccgccccgggcaccggcctggtcgacatgtcgagggacaggaacattccgcgcagccccaccagccccggtgagggattcgtcaatttcgactacggctggttcggcgcccagacggaagcggacgccgacaagaccgtctggacccacggaaatcactatcacgcgcccaatggcagcctgggtgccatgcatgtctacgagagcaagttccgcaactggtccgagggttactcggactgggaccgcggagcctatgtgatcaccttcatccccaagagctggaacaccgcccccgacaaggtaaagcagggctggccgtga

SEQ ID NO: 33 - DNA, 1134 bp, Artificial Sequence
  S303K/F305W mutant
atggacaatggcgcgggggaagagacgaagtcctacgccgaaacctaccgcctcacggcggatgacgtcgcgaacatcaacgcgctcaacgaaagcgctccggccgcttcgagcgccggcccgtcgttccgggcccccgactccgacgacagggtcacccctcccgccgagccgctcgacaggatgcccgacccgtaccgtccctcgtacggcagggccgagacggtcgtcaacaactacatacgcaagtggcagcaggtctacagccaccgcgacggcaggaagcagcagatgaccgaggagcagcgggagtggctgtcctacggctgcgtcggtgtcacctgggtcaattcgggtcagtacccgacgaacagactggccttcgcgtccttcgacgaggacaggttcaagaacgagctgaagaacggcaggccccggtccggcgagacgcgggcggagttcgagggccgcgtcgcgaaggagagcttcgacgaggagaagggcttccagcgggcgcgtgaggtggcgtccgtcatgaacagggccctggagaacgcccacgacgagagcgcttacctcgacaacctcaagaaggaactggcgaacggcaacgacgccctgcgcaacgaggacgcccgttccccgttctactcggcgctgcggaacacgccgtccttcaaggagcggaacggaggcaatcacgacccgtccaggatgaaggccgtcatctactcgaagcacttctggagcggccaggaccggtcgagttcggccgacaagaggaagtacggcgacccggacgccttccgccccgccccgggcaccggcctggtcgacatgtcgagggacaggaacattccgcgcagccccaccagccccggtgagggattcgtcaatttcgactacggctggttcggcgcccagacggaagcggacgccgacaagaccgtctggacccacggaaatcactatcacgcgcccaatggcagcctgggtgccatgcatgtctacgagagcaagttccgcaactggtccgagggttacaaggactgggaccgcggagcctatgtgatcaccttcatccccaagagctggaacaccgcccccgacaaggtaaagcagggctggccgtga

SEQ ID NO: 34 - DNA, 1134 bp, Artificial Sequence
  S303R/F305W mutant
atggacaatggcgcgggggaagagacgaagtcctacgccgaaacctaccgcctcacggcggatgacgtcgcgaacatcaacgcgctcaacgaaagcgctccggccgcttcgagcgccggcccgtcgttccgggcccccgactccgacgacagggtcacccctcccgccgagccgctcgacaggatgcccgacccgtaccgtccctcgtacggcagggccgagacggtcgtcaacaactacatacgcaagtggcagcaggtctacagccaccgcgacggcaggaagcagcagatgaccgaggagcagcgggagtggctgtcctacggctgcgtcggtgtcacctgggtcaattcgggtcagtacccgacgaacagactggccttcgcgtccttcgacgaggacaggttcaagaacgagctgaagaacggcaggccccggtccggcgagacgcgggcggagttcgagggccgcgtcgcgaaggagagcttcgacgaggagaagggcttccagcgggcgcgtgaggtggcgtccgtcatgaacagggccctggagaacgcccacgacgagagcgcttacctcgacaacctcaagaaggaactggcgaacggcaacgacgccctgcgcaacgaggacgcccgttccccgttctactcggcgctgcggaacacgccgtccttcaaggagcggaacggaggcaatcacgacccgtccaggatgaaggccgtcatctactcgaagcacttctggagcggccaggaccggtcgagttcggccgacaagaggaagtacggcgacccggacgccttccgccccgccccgggcaccggcctggtcgacatgtcgagggacaggaacattccgcgcagccccaccagccccggtgagggattcgtcaatttcgactacggctggttcggcgcccagacggaagcggacgccgacaagaccgtctggacccacggaaatcactatcacgcgcccaatggcagcctgggtgccatgcatgtctacgagagcaagttccgcaactggtccgagggttacagggactgggaccgcggagcctatgtgatcaccttcatccccaagagctggaacaccgcccccgacaaggtaaagcagggctggccgtga

SEQ ID NO: 35 - DNA, 1134 bp, Artificial Sequence
  R5H mutant
atggacaatggcgcgggggaagagacgaagtcctacgccgaaacctaccgcctcacggcggatgacgtcgcgaacatcaacgcgctcaacgaaagcgctccggccgcttcgagcgccggcccgtcgttccgggcccccgactccgacgaccacgtcacccctcccgccgagccgctcgacaggatgcccgacccgtaccgtccctcgtacggcagggccgagacggtcgtcaacaactacatacgcaagtggcagcaggtctacagccaccgcgacggcaggaagcagcagatgaccgaggagcagcgggagtggctgtcctacggctgcgtcggtgtcacctgggtcaattcgggtcagtacccgacgaacagactggccttcgcgtccttcgacgaggacaggttcaagaacgagctgaagaacggcaggccccggtccggcgagacgcgggcggagttcgagggccgcgtcgcgaaggagagcttcgacgaggagaagggcttccagcgggcgcgtgaggtggcgtccgtcatgaacagggccctggagaacgcccacgacgagagcgcttacctcgacaacctcaagaaggaactggcgaacggcaacgacgccctgcgcaacgaggacgcccgttccccgttctactcggcgctgcggaacacgccgtccttcaaggagcggaacggaggcaatcacgacccgtccaggatgaaggccgtcatctactcgaagcacttctggagcggccaggaccggtcgagttcggccgacaagaggaagtacggcgacccggacgccttccgccccgccccgggcaccggcctggtcgacatgtcgagggacaggaacattccgcgcagccccaccagccccggtgagggattcgtcaatttcgactacggctggttcggcgcccagacggaagcggacgccgacaagaccgtctggacccacggaaatcactatcacgcgcccaatggcagcctgggtgccatgcatgtctacgagagcaagttccgcaactggtccgagggttactcggacttcgaccgcggagcctatgtgatcaccttcatccccaagagctggaacaccgcccccgacaaggtaaagcagggctggccgtga

SEQ ID NO: 36 - DNA, 1134 bp, Artificial Sequence
  V6D mutant
atggacaatggcgcgggggaagagacgaagtcctacgccgaaacctaccgcctcacggcggatgacgtcgcgaacatcaacgcgctcaacgaaagcgctccggccgcttcgagcgccggcccgtcgttccgggcccccgactccgacgacagggacacccctcccgccgagccgctcgacaggatgcccgacccgtaccgtccctcgtacggcagggccgagacggtcgtcaacaactacatacgcaagtggcagcaggtctacagccaccgcgacggcaggaagcagcagatgaccgaggagcagcgggagtggctgtcctacggctgcgtcggtgtcacctgggtcaattcgggtcagtacccgacgaacagactggccttcgcgtccttcgacgaggacaggttcaagaacgagctgaagaacggcaggccccggtccggcgagacgcgggcggagttcgagggccgcgtcgcgaaggagagcttcgacgaggagaagggcttccagcgggcgcgtgaggtggcgtccgtcatgaacagggccctggagaacgcccacgacgagagcgcttacctcgacaacctcaagaaggaactggcgaacggcaacgacgccctgcgcaacgaggacgcccgttccccgttctactcggcgctgcggaacacgccgtccttcaaggagcggaacggaggcaatcacgacccgtccaggatgaaggccgtcatctactcgaagcacttctggagcggccaggaccggtcgagttcggccgacaagaggaagtacggcgacccggacgccttccgccccgccccgggcaccggcctggtcgacatgtcgagggacaggaacattccgcgcagccccaccagccccggtgagggattcgtcaatttcgactacggctggttcggcgcccagacggaagcggacgccgacaagaccgtctggacccacggaaatcactatcacgcgcccaatggcagcctgggtgccatgcatgtctacgagagcaagttccgcaactggtccgagggttactcggacttcgaccgcggagcctatgtgatcaccttcatccccaagagctggaacaccgcccccgacaaggtaaagcagggctggccgtga

SEQ ID NO: 37 - DNA, 1134 bp, Artificial Sequence
  W59T mutant
atggacaatggcgcgggggaagagacgaagtcctacgccgaaacctaccgcctcacggcggatgacgtcgcgaacatcaacgcgctcaacgaaagcgctccggccgcttcgagcgccggcccgtcgttccgggcccccgactccgacgacagggtcacccctcccgccgagccgctcgacaggatgcccgacccgtaccgtccctcgtacggcagggccgagacggtcgtcaacaactacatacgcaagtggcagcaggtctacagccaccgcgacggcaggaagcagcagatgaccgaggagcagcgggagaccctgtcctacggctgcgtcggtgtcacctgggtcaattcgggtcagtacccgacgaacagactggccttcgcgtccttcgacgaggacaggttcaagaacgagctgaagaacggcaggccccggtccggcgagacgcgggcggagttcgagggccgcgtcgcgaaggagagcttcgacgaggagaagggcttccagcgggcgcgtgaggtggcgtccgtcatgaacagggccctggagaacgcccacgacgagagcgcttacctcgacaacctcaagaaggaactggcgaacggcaacgacgccctgcgcaacgaggacgcccgttccccgttctactcggcgctgcggaacacgccgtccttcaaggagcggaacggaggcaatcacgacccgtccaggatgaaggccgtcatctactcgaagcacttctggagcggccaggaccggtcgagttcggccgacaagaggaagtacggcgacccggacgccttccgccccgccccgggcaccggcctggtcgacatgtcgagggacaggaacattccgcgcagccccaccagccccggtgagggattcgtcaatttcgactacggctggttcggcgcccagacggaagcggacgccgacaagaccgtctggacccacggaaatcactatcacgcgcccaatggcagcctgggtgccatgcatgtctacgagagcaagttccgcaactggtccgagggttactcggacttcgaccgcggagcctatgtgatcaccttcatccccaagagctggaacaccgcccccgacaaggtaaagcagggctggccgtga

SEQ ID NO: 38 - DNA, 1134 bp, Artificial Sequence
  S61G mutant
atggacaatggcgcgggggaagagacgaagtcctacgccgaaacctaccgcctcacggcggatgacgtcgcgaacatcaacgcgctcaacgaaagcgctccggccgcttcgagcgccggcccgtcgttccgggcccccgactccgacgacagggtcacccctcccgccgagccgctcgacaggatgcccgacccgtaccgtccctcgtacggcagggccgagacggtcgtcaacaactacatacgcaagtggcagcaggtctacagccaccgcgacggcaggaagcagcagatgaccgaggagcagcgggagtggctgggctacggctgcgtcggtgtcacctgggtcaattcgggtcagtacccgacgaacagactggccttcgcgtccttcgacgaggacaggttcaagaacgagctgaagaacggcaggccccggtccggcgagacgcgggcggagttcgagggccgcgtcgcgaaggagagcttcgacgaggagaagggcttccagcgggcgcgtgaggtggcgtccgtcatgaacagggccctggagaacgcccacgacgagagcgcttacctcgacaacctcaagaaggaactggcgaacggcaacgacgccctgcgcaacgaggacgcccgttccccgttctactcggcgctgcggaacacgccgtccttcaaggagcggaacggaggcaatcacgacccgtccaggatgaaggccgtcatctactcgaagcacttctggagcggccaggaccggtcgagttcggccgacaagaggaagtacggcgacccggacgccttccgccccgccccgggcaccggcctggtcgacatgtcgagggacaggaacattccgcgcagccccaccagccccggtgagggattcgtcaatttcgactacggctggttcggcgcccagacggaagcggacgccgacaagaccgtctggacccacggaaatcactatcacgcgcccaatggcagcctgggtgccatgcatgtctacgagagcaagttccgcaactggtccgagggttactcggacttcgaccgcggagcctatgtgatcaccttcatccccaagagctggaacaccgcccccgacaaggtaaagcagggctggccgtga

SEQ ID NO: 39 - DNA, 1134 bp, Artificial Sequence
  S61R mutant
atggacaatggcgcgggggaagagacgaagtcctacgccgaaacctaccgcctcacggcggatgacgtcgcgaacatcaacgcgctcaacgaaagcgctccggccgcttcgagcgccggcccgtcgttccgggcccccgactccgacgacagggtcacccctcccgccgagccgctcgacaggatgcccgacccgtaccgtccctcgtacggcagggccgagacggtcgtcaacaactacatacgcaagtggcagcaggtctacagccaccgcgacggcaggaagcagcagatgaccgaggagcagcgggagtggctgaggtacggctgcgtcggtgtcacctgggtcaattcgggtcagtacccgacgaacagactggccttcgcgtccttcgacgaggacaggttcaagaacgagctgaagaacggcaggccccggtccggcgagacgcgggcggagttcgagggccgcgtcgcgaaggagagcttcgacgaggagaagggcttccagcgggcgcgtgaggtggcgtccgtcatgaacagggccctggagaacgcccacgacgagagcgcttacctcgacaacctcaagaaggaactggcgaacggcaacgacgccctgcgcaacgaggacgcccgttccccgttctactcggcgctgcggaacacgccgtccttcaaggagcggaacggaggcaatcacgacccgtccaggatgaaggccgtcatctactcgaagcacttctggagcggccaggaccggtcgagttcggccgacaagaggaagtacggcgacccggacgccttccgccccgccccgggcaccggcctggtcgacatgtcgagggacaggaacattccgcgcagccccaccagccccggtgagggattcgtcaatttcgactacggctggttcggcgcccagacggaagcggacgccgacaagaccgtctggacccacggaaatcactatcacgcgcccaatggcagcctgggtgccatgcatgtctacgagagcaagttccgcaactggtccgagggttactcggacttcgaccgcggagcctatgtgatcaccttcatccccaagagctggaacaccgcccccgacaaggtaaagcagggctggccgtga

SEQ ID NO: 40 - DNA, 1134 bp, Artificial Sequence
  M288F mutant
atggacaatggcgcgggggaagagacgaagtcctacgccgaaacctaccgcctcacggcggatgacgtcgcgaacatcaacgcgctcaacgaaagcgctccggccgcttcgagcgccggcccgtcgttccgggcccccgactccgacgacagggtcacccctcccgccgagccgctcgacaggatgcccgacccgtaccgtccctcgtacggcagggccgagacggtcgtcaacaactacatacgcaagtggcagcaggtctacagccaccgcgacggcaggaagcagcagatgaccgaggagcagcgggagtggctgtcctacggctgcgtcggtgtcacctgggtcaattcgggtcagtacccgacgaacagactggccttcgcgtccttcgacgaggacaggttcaagaacgagctgaagaacggcaggccccggtccggcgagacgcgggcggagttcgagggccgcgtcgcgaaggagagcttcgacgaggagaagggcttccagcgggcgcgtgaggtggcgtccgtcatgaacagggccctggagaacgcccacgacgagagcgcttacctcgacaacctcaagaaggaactggcgaacggcaacgacgccctgcgcaacgaggacgcccgttccccgttctactcggcgctgcggaacacgccgtccttcaaggagcggaacggaggcaatcacgacccgtccaggatgaaggccgtcatctactcgaagcacttctggagcggccaggaccggtcgagttcggccgacaagaggaagtacggcgacccggacgccttccgccccgccccgggcaccggcctggtcgacatgtcgagggacaggaacattccgcgcagccccaccagccccggtgagggattcgtcaatttcgactacggctggttcggcgcccagacggaagcggacgccgacaagaccgtctggacccacggaaatcactatcacgcgcccaatggcagcctgggtgccttccatgtctacgagagcaagttccgcaactggtccgagggttactcggacttcgaccgcggagcctatgtgatcaccttcatccccaagagctggaacaccgcccccgacaaggtaaagcagggctggccgtga

SEQ ID NO: 41 - DNA, 1134 bp, Artificial Sequence
  M288L mutant
atggacaatggcgcgggggaagagacgaagtcctacgccgaaacctaccgcctcacggcggatgacgtcgcgaacatcaacgcgctcaacgaaagcgctccggccgcttcgagcgccggcccgtcgttccgggcccccgactccgacgacagggtcacccctcccgccgagccgctcgacaggatgcccgacccgtaccgtccctcgtacggcagggccgagacggtcgtcaacaactacatacgcaagtggcagcaggtctacagccaccgcgacggcaggaagcagcagatgaccgaggagcagcgggagtggctgtcctacggctgcgtcggtgtcacctgggtcaattcgggtcagtacccgacgaacagactggccttcgcgtccttcgacgaggacaggttcaagaacgagctgaagaacggcaggccccggtccggcgagacgcgggcggagttcgagggccgcgtcgcgaaggagagcttcgacgaggagaagggcttccagcgggcgcgtgaggtggcgtccgtcatgaacagggccctggagaacgcccacgacgagagcgcttacctcgacaacctcaagaaggaactggcgaacggcaacgacgccctgcgcaacgaggacgcccgttccccgttctactcggcgctgcggaacacgccgtccttcaaggagcggaacggaggcaatcacgacccgtccaggatgaaggccgtcatctactcgaagcacttctggagcggccaggaccggtcgagttcggccgacaagaggaagtacggcgacccggacgccttccgccccgccccgggcaccggcctggtcgacatgtcgagggacaggaacattccgcgcagccccaccagccccggtgagggattcgtcaatttcgactacggctggttcggcgcccagacggaagcggacgccgacaagaccgtctggacccacggaaatcactatcacgcgcccaatggcagcctgggtgccctgcatgtctacgagagcaagttccgcaactggtccgagggttactcggacttcgaccgcggagcctatgtgatcaccttcatccccaagagctggaacaccgcccccgacaaggtaaagcagggctggccgtga

SEQ ID NO: 42 - DNA, 1134 bp, Artificial Sequence
  M288Y mutant
atggacaatggcgcgggggaagagacgaagtcctacgccgaaacctaccgcctcacggcggatgacgtcgcgaacatcaacgcgctcaacgaaagcgctccggccgcttcgagcgccggcccgtcgttccgggcccccgactccgacgacagggtcacccctcccgccgagccgctcgacaggatgcccgacccgtaccgtccctcgtacggcagggccgagacggtcgtcaacaactacatacgcaagtggcagcaggtctacagccaccgcgacggcaggaagcagcagatgaccgaggagcagcgggagtggctgtcctacggctgcgtcggtgtcacctgggtcaattcgggtcagtacccgacgaacagactggccttcgcgtccttcgacgaggacaggttcaagaacgagctgaagaacggcaggccccggtccggcgagacgcgggcggagttcgagggccgcgtcgcgaaggagagcttcgacgaggagaagggcttccagcgggcgcgtgaggtggcgtccgtcatgaacagggccctggagaacgcccacgacgagagcgcttacctcgacaacctcaagaaggaactggcgaacggcaacgacgccctgcgcaacgaggacgcccgttccccgttctactcggcgctgcggaacacgccgtccttcaaggagcggaacggaggcaatcacgacccgtccaggatgaaggccgtcatctactcgaagcacttctggagcggccaggaccggtcgagttcggccgacaagaggaagtacggcgacccggacgccttccgccccgccccgggcaccggcctggtcgacatgtcgagggacaggaacattccgcgcagccccaccagccccggtgagggattcgtcaatttcgactacggctggttcggcgcccagacggaagcggacgccgacaagaccgtctggacccacggaaatcactatcacgcgcccaatggcagcctgggtgcctaccatgtctacgagagcaagttccgcaactggtccgagggttactcggacttcgaccgcggagcctatgtgatcaccttcatccccaagagctggaacaccgcccccgacaaggtaaagcagggctggccgtga

SEQ ID NO: 43 - DNA, 1134 bp, Artificial Sequence
  V290I mutant
atggacaatggcgcgggggaagagacgaagtcctacgccgaaacctaccgcctcacggcggatgacgtcgcgaacatcaacgcgctcaacgaaagcgctccggccgcttcgagcgccggcccgtcgttccgggcccccgactccgacgacagggtcacccctcccgccgagccgctcgacaggatgcccgacccgtaccgtccctcgtacggcagggccgagacggtcgtcaacaactacatacgcaagtggcagcaggtctacagccaccgcgacggcaggaagcagcagatgaccgaggagcagcgggagtggctgtcctacggctgcgtcggtgtcacctgggtcaattcgggtcagtacccgacgaacagactggccttcgcgtccttcgacgaggacaggttcaagaacgagctgaagaacggcaggccccggtccggcgagacgcgggcggagttcgagggccgcgtcgcgaaggagagcttcgacgaggagaagggcttccagcgggcgcgtgaggtggcgtccgtcatgaacagggccctggagaacgcccacgacgagagcgcttacctcgacaacctcaagaaggaactggcgaacggcaacgacgccctgcgcaacgaggacgcccgttccccgttctactcggcgctgcggaacacgccgtccttcaaggagcggaacggaggcaatcacgacccgtccaggatgaaggccgtcatctactcgaagcacttctggagcggccaggaccggtcgagttcggccgacaagaggaagtacggcgacccggacgccttccgccccgccccgggcaccggcctggtcgacatgtcgagggacaggaacattccgcgcagccccaccagccccggtgagggattcgtcaatttcgactacggctggttcggcgcccagacggaagcggacgccgacaagaccgtctggacccacggaaatcactatcacgcgcccaatggcagcctgggtgccatgcatatctacgagagcaagttccgcaactggtccgagggttactcggacttcgaccgcggagcctatgtgatcaccttcatccccaagagctggaacaccgcccccgacaaggtaaagcagggctggccgtga

SEQ ID NO: 44 - protein, 410 aa, Streptomyces mobaraensis
MSQRGRTLVFAALGAVMCTTALMPSAGAATGSGSGSGTGEEKRSYAETHRLTADDVDDINALNESAPAASSAGPSFRAPDSDERVTPPAEPLDRMPDPYRPSYGRAETIVNNYIRKWQQVYSHRDGRKQQMTEEQREWLSYGCVGVTWVNSGQYPTNRLAFAFFDEDKYKNELKNGRPRSGETRAEFEGRVAKDSFDEAKGFQRARDVASVMNKALENAHDEGAYLDNLKKELANGNDALRNEDARSPFYSALRNTPSFKDRNGGNHDPSKMKAVIYSKHFWSGQDRSGSSDKRKYGDPEAFRPDRGTGLVDMSRDRNIPRSPTSPGESFVNFDYGWFGAQTEADADKTVWTHGNHYHAPNGSLGAMHVYESKFRNWSDGYSDFDRGAYVVTFVPKSWNTAPDKVTQGWP

SEQ ID NO: 45 - protein, 418 aa, Streptomyces albireticuli
MYKRPRFLTFAAAGAVICTAGFTPSVSQAAGGGDVVTKGSYAETHGLTADDIKNINALNERAMAVGQPDKPPTETPPSAGPPSRTPDSDDDRETPPAEPLDRMPDAYRAYGGRATTVVNNYIRKWQQVYSHRDGKKQQMTEEQREMLSYGCVGVTWVNSGLYPTNRLAFASFDENKYKNDLTNTSPRPGETRAEFEGRIAKGSFDERKGFKRARDVASVMNKALENAHDEGTYISNLKADLTNKNDALLHEDSRSNFYSALRNTPSFRERDGGNYDPSKMKAVIYSKHFWSGQDQRGSSDKRKYGDAEAFRPDQGTGLVDMSRDRNIPRSPTSPGEGWVNFDYGWFGAQTEADADKTTWTHGDHYHAPNSDLGPMHVHESKFRNWSAGYADFDRGAYVITFIPKSWNTAPGKVEQGWP

SEQ ID NO: 46 - protein, 400 aa, Streptomyces luteireticuli
FATVSAVVCTAGLMPSVSQAAGNREGEEKPSYAETHGLTAADVENINALNERALTLGRHGATPSFRAPDSANVRETPPAEPLDRMPDAYRARGGRATTVVNNYIRKWQQVYSHLDGKKQQMTEEQREKLSYGCVGVTWVNSGPYPTNRLAFSFFDEDKYKNDLKNTRPLAGETRAEFEGRIAKASFDEGKGFKRARDVASIMNKALENAHDEGAYLDKLKTELTNNNDALLHEDSRSNFYSALRNTPSFKERDGGNYDPSRMKAVIYSKHFWSGQDQRGSSDKRKYGDPEAFRPDRGTGLVDMSKDRNIPRSPANPGEGWVNFDYGWFGAQTEADADKTIWTHGDHYHAPNGDLGPMHVYESKFRNWSAGYADFDRGTYMIALIPKSWNTAPAKVKQGWP

SEQ ID NO: 47 - protein, 418 aa, Streptomyces cinnamoneus
MHQRRRLLAFATVGAFICTAGLTPSVSQAAGSGDGKEKGSYAETHGLTADDVKNINALNESALTLGQPGKPPAELPPSASASSRAPASDDDRVTPPAEPLDRMPDAYRAYGGRATTVVNNYIRKWQQVYSHRDGKKQQMTEEQREKLSYGCVGVTWVNSGPYPTNKLAFAFFDENKYKNDLKNTSPRPGETRAEFEGRIAKDSFDEGKGFKRARDVASIMNKALENAHDEGTYIDHLKTELTNKNDALLHEDSRSNFYSALRNTPSFKERDGGNYDPSKMKAVIYSKHFWSGQDQRGPSDKRKYGDPEAFRPAQGTGLVDMSKDKSIPRSPANPGEGWVNFDYGWFGAQTEADADNTTWTHGDHYHAPNSDLGPMHVHESKFRKWSAGYEDFDRGSYVITFIPKSWNTAPAAVKQGWP

SEQ ID NO: 48 - protein, 418 aa, Streptomyces platensis
MYKRRSLLAFATVSAAIFTAGVMPSVSHAASGGDGETEGSYAETHGLTAEDVKNINALNKRALTAGQPGNSLAELPPSVSALFRAPDAADERVTPPAEPLNRMPDAYRAYGGRATTVVNNYIRKWQQVYSHRDGIQQQMTEEQREKLSYGCVGVTWVNSGPYPTNKLAFAFFDEDKYKSDLENSRPRPNETQAEFEGRIVKDSFDEGKGFKRARDVASVMNKALDSAHDEGTYIDNLKKELANKNDALRYEDSRSNFYSALRNTPSFKERDGGNYDPSKMKAVVYSKHFWSGQDQRGSSDKRKYGDPDAFRPDQGTGLVDMSKDRNIPRSPARPGESWVNFDYGWFGAQTEADADKTIWTHANHYHAPNGGVGPMNVYESKFRNWSAGYADFDRGTYVITFIPKSWNTAPAEVKQGWS

SEQ ID NO: 49 - protein, 418 aa, Streptomyces hygroscopicus
MYKRRSLLAFATVSAAIFTAGVMPSVSHAASGGDGEREGSYAETHGLTAEDVKNINALNKRALTAGQPGNSLAELPPSVSALFRAPDAADERVTPPAEPLNRMPDAYRAYGGRATTVVNNYIRKWQQVYSHRDGIQQQMTEEQREKLSYGCVGVTWVNSGPYPTNKLAFAFFDEDKYKSDLENSRPRPNETQAEFEGRIVKDSFDEGKGFKRARDVASIMNKALDSAHDEGTYIDNLKKELANKNDALRYEDSRSNFYSALRNTPSFKERDGGNYDPSKMKAVVYSKHFWSGQDQRGSSDKRKYGDPDAFRPDQGTGLVDMSKDRNIPRSPARPGESWVNFDYGWFGAQTEADADKTIWTHANHYHAPNGGVGPMNVYESKFRNWSAGYADFDRGTYVITFIPKSWNTAPAEVKQGWS

SEQ ID NO: 50 - DNA, 1134 bp, Streptomyces mobaraensis
atggacaatggcgcgggggaagagacgaagtcctacgccgaaacctaccgcctcacggcggatgacgtcgcgaacatcaacgcgctcaacgaaagcgctccggccgcttcgagcgccggcccgtcgttccgggcccccgactccgacgacagggtcacccctcccgccgagccgctcgacaggatgcccgacccgtaccgtccctcgtacggcagggccgagacggtcgtcaacaactacatacgcaagtggcagcaggtctacagccaccgcgacggcaggaagcagcagatgaccgaggagcagcgggagtggctgtcctacggctgcgtcggtgtcacctgggtcaattcgggtcagtacccgacgaacagactggccttcgcgtccttcgacgaggacaggttcaagaacgagctgaagaacggcaggccccggtccggcgagacgcgggcggagttcgagggccgcgtcgcgaaggagagcttcgacgaggagaagggcttccagcgggcgcgtgaggtggcgtccgtcatgaacagggccctggagaacgcccacgacgagagcgcttacctcgacaacctcaagaaggaactggcgaacggcaacgacgccctgcgcaacgaggacgcccgttccccgttctactcggcgctgcggaacacgccgtccttcaaggagcggaacggaggcaatcacgacccgtccaggatgaaggccgtcatctactcgaagcacttctggagcggccaggaccggtcgagttcggccgacaagaggaagtacggcgacccggacgccttccgccccgccccgggcaccggcctggtcgacatgtcgagggacaggaacattccgcgcagccccaccagccccggtgagggattcgtcaatttcgactacggctggttcggcgcccagacggaagcggacgccgacaagaccgtctggacccacggaaatcactatcacgcgcccaatggcagcctgggtgccatgcatgtctacgagagcaagttccgcaactggtccgagggttactcggacttcgaccgcggagcctatgtgatcaccttcatccccaagagctggaacaccgcccccgacaaggtaaagcagggctggccgtga

SEQ ID NO: 51 - protein, 31 aa, Streptomyces mobaraensis
MRIRRRALVFATMSAVLCTAGFMPSAGEAAA

SEQ ID NO: 52 - protein, 45 aa, Streptomyces mobaraensis
DNGAGEETKSYAETYRLTADDVANINALNESAPAASSAGPSFRAP

SEQ ID NO: 53 - DNA, 93 bp, Streptomyces mobaraensis
atgcgcatacgccggagagctctcgtcttcgccactatgagtgcggtgttatgcaccgccggattcatgccgtcggccggcgaggccgccgcc

SEQ ID NO: 54 - DNA, 135 bp, Streptomyces mobaraensis
gacaatggcgcgggggaagagacgaagtcctacgccgaaacctaccgcctcacggcggatgacgtcgcgaacatcaacgcgctcaacgaaagcgctccggccgcttcgagcgccggcccgtcgttccgggccccc